European Patent Application EP 4 707 294 A1, published March 11, 2026. Title: Microorganism of Corynebacterium genus producing L-glutamic acid and method for producing L-glutamic acid using the same. Applicant: DAESANG CORPORATION. The sequence listing filed with the application follows.

SEQUENCE LISTING (9 sequences)

SEQ ID NO: 1 - DNA, 1527 bp, synthetic construct
  source 1..1527: mol_type = other DNA
atgacggacatcaaggccacatcaagtacatcggccactacagcaccaacagcaggccgaccagcgcgtcgacttggacaaatctccctcgtcgcctgtctcggcggactcctcttcggctatgacaccggtgtcgccaacggcgccgaaggccacatggcacaagaactcggactcaacgtgctgcaactcggcgttgtcatcagttcactggttttcgctgcagcctttggtgcgctgttcgctgggcgtatctcggacgaaatcgggcgtcgaaaagcaattatcactttgtccgtgctgttcttcctcggatcaatcctcgtcgtattctcccccgccggtgagctggggcagttctacggaccaggatttgccaccttggtcaccgggcgcatcatgttgggtctcgcggttggcggcgcctccacagtagttccggtgtacctcgctgaactcgcaccactagaaatccgcggctccctgaccggccgaaacgagcttgctatcgtcaccggccagctgcttgccttcgtgatcaacgcgcttatcgccgtcaccctacacggagttattgatggaatctggcgcatcatgttcgccgtctgtgccctccctgccgtcgccctcttcctcggcatgctgcggatgccggaatcaccacgctggctggtcaaccaggggcgttacgacgacgcccgccgcgtcatggagactgtccgtacccctgagcgtgcgaaagtcgaaatggatgaaatcatcgcggtgcactctgaaaacaatgcggcacttcctggtgttaagcagtctgcgggccaggcttcaggccaggtttctagcaagcacacccacatgtccatcggcgaagtcctcagcaacaaatggctggttcgtctgctcatcgccggcatcggtgttgcagttgcccagcagctcaccggcatcaacgccatcatgtactacggaacccgcgtcctcgaggaatccggcatgagcgcagaaatggctgtggttgccaacattgctttcggtgccgttgccgtcatcggtggactgatcgcactgcgcaacatggaccgcctggatcgccgcaccaccttcatcatcggcctgtcactgaccaccaccttccaccttttgatcgcagctgctggcactctccttccagaaggtaactccattcgaccattcgccatcatgatccttgttgttgggttcgtgctctccatgcagaccttcctcaacgttgcagtgtgggtgtggctggcgaaaatcttcccagtccgaatgaagggtatcggcaccggtatctcggtattctgcggttggggcatcaatggcgtcctagcgttgttcttcccagcactggtctccggcgtgggtatcaccttctccttccttatcttcgcagtcgtcggagtcattgccctggcgttcgtcaccaagtttgttcctgaaacccgtggccgctcacttgaagaactcgaccacgcagcattcaccggccagatcttcaagaaggcttaa

SEQ ID NO: 2 - protein, 508 aa, synthetic construct
MTDIKATSSTSATTAPTAGRPARRLGQISLVACLGGLLFGYDTGVANGAEGHMAQELGLNVLQLGVVISSLVFAAAFGALFAGRISDEIGRRKAIITLSVLFFLGSILVVFSPAGELGQFYGPGFATLVTGRIMLGLAVGGASTVVPVYLAELAPLEIRGSLTGRNELAIVTGQLLAFVINALIAVTLHGVIDGIWRIMFAVCALPAVALFLGMLRMPESPRWLVNQGRYDDARRVMETVRTPERAKVEMDEIIAVHSENNAALPGVKQSAGQASGQVSSKHTHMSIGEVLSNKWLVRLLIAGIGVAVAQQLTGINAIMYYGTRVLEESGMSAEMAVVANIAFGAVAVIGGLIALRNMDRLDRRTTFIIGLSLTTTFHLLIAAAGTLLPEGNSIRPFAIMILVVGFVLSMQTFLNVAVWVWLAKIFPVRMKGIGTGISVFCGWGINGVLALFFPALVSGVGITFSFLIFAVVGVIALAFVTKFVPETRGRSLEELDHAAFTGQIFKKA

SEQ ID NO: 3 - DNA, 1527 bp, Corynebacterium glutamicum
  source 1..1527: mol_type = genomic DNA
atgacggacatcaaggccacatcaagtacatcggccactacagcaccaacagcaggccgaccagcgcgtcgacttggacaaatctccctcgtcgcctgtctcggcggactcctcttcggctatgacaccggtgtcgccaacggcgccgaaggccacatggcacaagaactcggactcaacgtgctgcaactcggcgttgtcatcagttcactggttttcgctgcagcctttggtgcgctgttcgctgggcgtatctcggacgaaatcgggcgtcgaaaagcaattatcactttgtccgtgctgttcttcctcggatcaatcctcgtcgtattctcccccgccggtgagctggggcagttctacggaccaggatttgccaccttggtcaccgggcgcatcatgttgggtctcgcggttggcggcgcctccacagtagttccggtgtacctcgctgaactcgcaccactagaaatccgcggctccctgaccggccgaaacgagcttgctatcgtcaccggccagctgcttgccttcgtgatcaacgcgcttatcgccgtcaccctacacggagttattgatggaatctggcgcatcatgttcgccgtctgtgccctccctgccgtcgccctcttcctcggcatgctgcggatgccggaatcaccacgctggctggtcaaccaggggcgttacgacgacgcccgccgcgtcatggagactgtccgtacccctgagcgtgcgaaagtcgaaatggatgaaatcatcgcggtgcactctgaaaacaatgcggcacttcctggtgttaagcagtctgcgggccaggcttcaggccaggtttctagcaagcacacccacatgtccatcggcgaagtcctcagcaacaaatggctggttcgtctgctcatcgccggcatcggtgttgcagttgcccagcagctcaccggcatcaacgccatcatgtactacggaacccgcgtcctcgaggaatccggcatgagcgcagaaatggctgtggttgccaacattgctttcggtgccgttgccgtcatcggtggactgatcgcactgcgcaacatggaccgcctggatcgccgcaccaccttcatcatcggcctgtcactgaccaccaccttccaccttttgatcgcagctgctggcactctccttccagaaggtaactccattcgaccattcgccatcatgatccttgttgttgggttcgtgctctccatgcagaccttcctcaacgttgcagtgtgggtgtggctggcggaaatcttcccagtccgaatgaagggtatcggcaccggtatctcggtattctgcggttggggcatcaatggcgtcctagcgttgttcttcccagcactggtctccggcgtgggtatcaccttctccttccttatcttcgcagtcgtcggagtcattgccctggcgttcgtcaccaagtttgttcctgaaacccgtggccgctcacttgaagaactcgaccacgcagcattcaccggccagatcttcaagaaggcttaa

SEQ ID NO: 4 - protein, 508 aa, Corynebacterium glutamicum
MTDIKATSSTSATTAPTAGRPARRLGQISLVACLGGLLFGYDTGVANGAEGHMAQELGLNVLQLGVVISSLVFAAAFGALFAGRISDEIGRRKAIITLSVLFFLGSILVVFSPAGELGQFYGPGFATLVTGRIMLGLAVGGASTVVPVYLAELAPLEIRGSLTGRNELAIVTGQLLAFVINALIAVTLHGVIDGIWRIMFAVCALPAVALFLGMLRMPESPRWLVNQGRYDDARRVMETVRTPERAKVEMDEIIAVHSENNAALPGVKQSAGQASGQVSSKHTHMSIGEVLSNKWLVRLLIAGIGVAVAQQLTGINAIMYYGTRVLEESGMSAEMAVVANIAFGAVAVIGGLIALRNMDRLDRRTTFIIGLSLTTTFHLLIAAAGTLLPEGNSIRPFAIMILVVGFVLSMQTFLNVAVWVWLAEIFPVRMKGIGTGISVFCGWGINGVLALFFPALVSGVGITFSFLIFAVVGVIALAFVTKFVPETRGRSLEELDHAAFTGQIFKKA

SEQ ID NO: 5 - DNA, 5719 bp, synthetic construct
  source 1..5719: mol_type = other DNA
tgccgcaagcactcagggcgcaagggctgctaaaggaagcggaacacgtagaaagccagtccgcagaaacggtgctgaccccggatgaatgtcagctactgggctatctggacaagggaaaacgcaagcgcaaagagaaagcaggtagcttgcagtgggcttacatggcgatagctagactgggcggttttatggacagcaagcgaaccggaattgccagctggggcgccctctggtaaggttgggaagccctgcaaagtaaactggatggctttcttgccgccaaggatctgatggcgcaggggatcaagatctgatcaagagacaggatgaggatcgtttcgcatgattgaacaagatggattgcacgcaggttctccggccgcttgggtggagaggctattcggctatgactgggcacaacagacaatcggctgctctgatgccgccgtgttccggctgtcagcgcaggggcgcccggttctttttgtcaagaccgacctgtccggtgccctgaatgaactccaagacgaggcagcgcggctatcgtggctggccacgacgggcgttccttgcgcagctgtgctcgacgttgtcactgaagcgggaagggactggctgctattgggcgaagtgccggggcaggatctcctgtcatctcaccttgctcctgccgagaaagtatccatcatggctgatgcaatgcggcggctgcatacgcttgatccggctacctgcccattcgaccaccaagcgaaacatcgcatcgagcgagcacgtactcggatggaagccggtcttgtcgatcaggatgatctggacgaagagcatcaggggctcgcgccagccgaactgttcgccaggctcaaggcgcggatgcccgacggcgaggatctcgtcgtgacccatggcgatgcctgcttgccgaatatcatggtggaaaatggccgcttttctggattcatcgactgtggccggctgggtgtggcggaccgctatcaggacatagcgttggctacccgtgatattgctgaagagcttggcggcgaatgggctgaccgcttcctcgtgctttacggtatcgccgctcccgattcgcagcgcatcgccttctatcgccttcttgacgagttcttctgagcgggactctggggttcgctagaggatcgatcctttttaacccatcacatatacctgccgttcactattatttagtgaaatgagatattatgatattttctgaattgtgattaaaaaggcaactttatgcccatgcaacagaaactataaaaaatacagagaatgaaaagaaacagatagattttttagttctttaggcccgtagtctgcaaatccttttatgattttctatcaaacaaaagaggaaaatagaccagttgcaatccaaacgagagtctaatagaatgaggtcgaaaagtaaatcgcgcgggtttgttactgataaagcaggcaagacctaaaatgtgtaaagggcaaagtgtatactttggcgtcaccccttacatattttaggtctttttttattgtgcgtaactaacttgccatcttcaaacaggagggctggaagaagcagaccgctaacacagtacataaaaaaggagacatgaacgatgaacatcaaaaagtttgcaaaacaagcaacagtattaacctttactaccgcactgctggcaggaggcgcaactcaagcgtttgcgaaagaaacgaaccaaaagccatataaggaaacatacggcatttcccatattacacgccatgatatgctgcaaatccctgaacagcaaaaaaatgaaaaatatcaagtttctgaatttgattcgtccacaattaaaaatatctcttctgcaaaaggcctggacgtttgggacagctggccattacaaaacgctgacggcactgtcgcaaactatcacggctaccacatcgtctttgcattagccggagatcctaaaaatgcggatgacacatcgatttacatgttctatcaaaaagtcggcgaaacttctattgacagctggaaaaacgctggccgcgtctttaaagacagcgacaaattcgatgcaaatgattctatcctaaaagaccaaacacaagaatggtcaggttcagccacatttacatctgacggaaaaatccgtttattctacactgatttctccggtaaacattacggcaaacaaacactgacaactgcacaagttaacgtatcagcatcagacagctctttgaacatcaacggtgtagaggattataaatcaatctttgacggtgacggaaaaacgtatcaaaatgtacagcagttcatcgatgaaggcaactacagctcaggcgacaaccatacgctgagagatcctcactacgtagaagataaaggccacaaatacttagtatttgaagcaaacactggaactgaagatggctaccaaggcgaagaatctttatttaacaaagcatactatggcaaaagcacatcattcttccgtcaagaaagtcaaaaacttctgcaaagcgataaaaaacgcacggctgagttagcaaacggcgctctcggtatgattgagctaaacgatgattacacactgaaaaaagtgatgaaaccgctgattgcatctaacacagtaacagatgaaattgaacgcgcgaacgtctttaaaatgaacggcaaatggtacctgttcactgactcccgcggatcaaaaatgacgattgacggcattacgtctaacgatatttacatgcttggttatgtttctaattctttaactggcccatacaagccgctgaacaaaactggccttgtgttaaaaatggatcttgatcctaacgatgtaacctttacttactcacacttcgctgtacctcaagcgaaaggaaacaatgtcgtgattacaagctatatgacaaacagaggattctacgcagacaaacaatcaacgtttgcgccgagcttcctgctgaacatcaaaggcaagaaaacatctgttgtcaaagacagcatccttgaacaaggacaattaacagttaacaaataaaaacgcaaaagaaaatgccgatgggtaccgagcgaaatgaccgaccaagcgacgcccaacctgccatcacgagatttcgattccaccgccgccttctatgaaaggttgggcttcggaatcgttttccgggacgccctcgcggacgtgctcatagtccacgacgcccgtgattttgtagccctggccgacggccagcaggtaggccgacaggctcatgccggccgccgccgccttttcctcaatcgctcttcgttcgtctggaaggcagtacaccttgataggtgggctgcccttcctggttggcttggtttcatcagccatccgcttgccctcatctgttacgccggcggtagccggccagcctcgcagagcaggattcccgttgagcaccgccaggtgcgaataagggacagtgaagaaggaacacccgctcgcgggtgggcctacttcacctatcctgcccggctgacgccgttggatacaccaaggaaagtctacacgaaccctttggcaaaatcctgtatatcgtgcgaaaaaggatggatataccgaaaaaatcgctataatgaccccgaagcagggttatgcagcggaaaagcgctgcttccctgctgttttgtggaatatctaccgactggaaacaggcaaatgcaggaaattactgaactgaggggacaggcgagagacgatgccaaagagctcctgaaaatctcgataactcaaaaaatacgcccggtagtgatcttatttcattatggtgaaagttggaacctcttacgtgccgatcaacgtctcattttcgccaaaagttggcccagggcttcccggtatcaacagggacaccaggatttatttattctgcgaagtgatcttccgtcacaggtatttattcggcgcaaagtgcgtcgggtgatgctgccaacttactgatttagtgtatgatggtgtttttgaggtgctccagtggcttctgtttctatcagctcctgaaaatctcgataactcaaaaaatacgcccggtagtgatcttatttcattatggtgaaagttggaacctcttacgtgccgatcaacgtctcattttcgccaaaagttggcccagggcttcccggtatcaacagggacaccaggatttatttattctgcgaagtgatcttccgtcacaggtatttattcggcgcaaagtgcgtcgggtgatgctgccaacttactgatttagtgtatgatggtgtttttgaggtgctccagtggcttctgtttctatcagggctggatgatcctccagcgcggggatctcatgctggagttcttcgcccaccccaaaaggatctaggtgaagatcctttttgataatctcatgaccaaaatcccttaacgtgagttttcgttccactgagcgtcagaccccgtagaaaagatcaaaggatcttcttgagatcctttttttctgcgcgtaatctgctgcttgcaaacaaaaaaaccaccgctaccagcggtggtttgtttgccggatcaagagctaccaactctttttccgaaggtaactggcttcagcagagcgcagataccaaatactgttcttctagtgtagccgtagttaggccaccacttcaagaactctgtagcaccgcctacatacctcgctctgctaatcctgttaccagtggctgctgccagtggcgataagtcgtgtcttaccgggttggactcaagacgatagttaccggataaggcgcagcggtcgggctgaacggggggttcgtgcacacagcccagcttggagcgaacgacctacaccgaactgagatacctacagcgtgagctatgagaaagcgccacgcttcccgaagggagaaaggcggacaggtatccggtaagcggcagggtcggaacaggagagcgcacgagggagcttccagggggaaacgcctggtatctttatagtcctgtcgggtttcgccacctctgacttgagcgtcgatttttgtgatgctcgtcaggggggcggagcctatggaaaaacgccagcaacgcggcctttttacggttcctggccttttgctggccttttgctcacatgttctttcctgcgttatcccctgattctgtggataaccgtattaccgcctttgagtgagctgataccgctcgccgcagccgaacgaccgagcgcagcgagtcagtgagcgaggaagcggaagagcgcccaatacgcaaaccgcctctccccgcgcgttggccgattcattaatgcagctggcacgacaggtttcccgactggaaagcgggcagtgagcgcaacgcaattaatgtgagttagctcactcattaggcaccccaggctttacactttatgcttccggctcgtatgttgtgtggaattgtgagcggataacaatttcacacaggaaacagctatgacatgattacgccaagcttgcatgcctgcaggtcgactctagaggatccccgggtaccgagctcgaattcactggccgtcgttttacaacgtcgtgactgggaaaaccctggcgttacccaacttaatcgccttgcagcacatccccctttcgccagctggcgtaatagcgaagaggcccgcaccgatcgcccttcccaacagttgcgcagcctgaatggcgaatggcgataagctagcttcacgc

SEQ ID NO: 6 - DNA, 19 bp, synthetic construct
  source 1..19: mol_type = other DNA
acaatgcggcacttcctgg

SEQ ID NO: 7 - DNA, 20 bp, synthetic construct
  source 1..20: mol_type = other DNA
ggaagattttcgccagccac

SEQ ID NO: 8 - DNA, 20 bp, synthetic construct
  source 1..20: mol_type = other DNA
gtggctggcgaaaatcttcc

SEQ ID NO: 9 - DNA, 19 bp, synthetic construct
  source 1..19: mol_type = other DNA
cgatctcattgtcggttgc